European Patent Application EP 4 809 831 A1, published September 23, 2026. Title: 락토바실러스 속 균주 및 한약재를 포함하는 병용 요법을 이용한 수면장애 예방 또는 개선용 조성물. Applicant: 주식회사 지아이바이옴. The sequence listing filed with the application follows.

SEQUENCE LISTING (3 sequences)

SEQ ID NO: 1 - RNA, 1441 nt, Lactobacillus fermentum
  source 1..1441: mol_type = rRNA
gcaagtcgaacgcgttggcccaattgattgatggtgcttgcacctgattgattttggtcgccaacgagtggcggacgggtgagtaacacgtaggtaacctgcccagaagcgggggacaacatttggaaacagatgctaataccgcataacaacgttgttcgcatgaacaacgcttaaaagatggcttctcgctatcacttctggatggacctgcggtgcattagcttgttggtggggtaatggcctaccaaggcgatgatgcatagccgagttgagagactgatcggccacaatgggactgagacacggcccatactcctacgggaggcagcagtagggaatcttccacaatgggcgcaagcctgatggagcaacaccgcgtgagtgaagaagggtttcggctcgtaaagctctgttgttaaagaagaacacgtatgagagtaactgttcatacgttgacggtatttaaccagaaagtcacggctaactacgtgccagcagccgcggtaatacgtaggtggcaagcgttatccggatttattgggcgtaaagagagtgcaggcggttttctaagtctgatgtgaaagccttcggcttaaccggagaagtgcatcggaaactggataacttgagtgcagaagagggtagtggaactccatgtgtagcggtggaatgcgtagatatatggaagaacaccagtggcgaaggcggctacctggtctgcaactgacgctgagactcgaaagcatgggtagcgaacaggattagataccctggtagtccatgccgtaaacgatgagtgctaggtgttggagggtttccgcccttcagtgccggagctaacgcattaagcactccgcctggggagtacgaccgcaaggttgaaactcaaaggaattgacgggggcccgcacaagcggtggagcatgtggtttaattcgaagctacgcgaagaaccttaccaggtcttgacatcttgcgccaaccctagagatagggcgtttccttcgggaacgcaatgacaggtggtgcatggtcgtcgtcagctcgtgtcgtgagatgttgggttaagtcccgcaacgagcgcaacccttgttactagttgccagcattaagttgggcactctagtgagactgccggtgacaaaccggaggaaggtggggacgacgtcagatcatcatgccccttatgacctgggctacacacgtgctacaatggacggtacaacgagtcgcgaactcgcgagggcaagcaaatctcttaaaaccgttctcagttcggactgcaggctgcaactcgcctgcacgaagtcggaatcgctagtaatcgcggatcagcatgccgcggtgaatacgttcccgggccttgtacacaccgcccgtcacaccatgagagtttgtaacacccaaagtcggtggggtaaccttttaggagccagcc

SEQ ID NO: 2 - RNA, 1447 nt, Lactobacillus fermentum
  source 1..1447: mol_type = rRNA
atacatgcaagtcgaacgcgttggcccaattgattgatggtgcttgcacctgattgattttggtcgccaacgagtggcggacgggtgagtaacacgtaggtaacctgcccagaagcgggggacaacatttggaaacagatgctaataccgcataacagcgttgttcgcatgaacaacgcttaaaagatggcttctcgctatcacttctggatggacctgcggtgcattagcttgttggtggggtaacggcctaccaaggcgatgatgcatagccgagttgagagactgatcggccacaatgggactgagacacggcccatactcctacgggaggcagcagtagggaatcttccacaatgggcgcaagcctgatggagcaacaccgcgtgagtgaagaagggtttcggctcgtaaagctctgttgttaaagaagaacacgtatgagagtaactgttcatacgttgacggtatttaaccagaaagtcacggctaactacgtgccagcagccgcggtaatacgtaggtggcaagcgttatccggatttattgggcgtaaagagagtgcaggcggttttctaagtctgatgtgaaagccttcggcttaaccggagaagtgcatcggaaactggataacttgagtgcagaagagggtagtggaactccatgtgtagcggtggaatgcgtagatatatggaagaacaccagtggcgaaggcggctacctggtctgcaactgacgctgagactcgaaagcatgggtagcgaacaggattagataccctggtagtccatgccgtaaacgatgagtgctaggtgttggagggtttccgcccttcagtgccggagctaacgcattaagcactccgcctggggagtacgaccgcaaggttgaaactcaaaggaattgacgggggcccgcacaagcggtggagcatgtggtttaattcgaagctacgcgaagaaccttaccaggtcttgacatcttgcgccaaccctagagatagggcgtttccttcgggaacgcaatgacaggtggtgcatggtcgtcgtcagctcgtgtcgtgagatgttgggttaagtcccgcaacgagcgcaacccttgttactagttgccagcattaagttgggcactctagtgagactgccggtgacaaaccggaggaaggtggggacgacgtcagatcatcatgccccttatgacctgggctacacacgtgctacaatggacggtacaacgagtcgcgaactcgcgagggcaagcaaatctcttaaaaccgttctcagttcggactgcaggctgcaactcgcctgcacgaagtcggaatcgctagtaatcgcggatcagcatgccgcggtgaatacgttcccgggccttgtacacaccgcccgtcacaccatgagagtttgtaacacccaaagtcggtggggtaaccttttaggagccagcc

SEQ ID NO: 3 - RNA, 1552 nt, Lactobacillus plantarum
  source 1..1552: mol_type = rRNA
agagtttgatcctggctcaggacgaacgctggcggcgtgcctaatacatgcaagtcgaacgaactctggtattgattggtgcttgcatcatgatttacatttgagtgagtggcgaactggtgagtaacacgtgggaaacctgcccagaagcgggggataacacctggaaacagatgctaataccgcataacaacttggaccgcatggtccgagtttgaaagatggctttggctatcacttttggatggtcccgcggcgtattagctagatggtggggtaacggctcaccatggcaatgatacgtagccgacctgagagggtaatcggccacattgggactgagacacggcccaaactcctacgggaggcagcagtagggaatcttccacaatggacgaaagtctgatggagcaacgccgcgtgagtgaagaagggtttcggctcgtaaaactctgttgttaaagaagaacatatctgagagtaactgttcaggtattgacggtatttaaccagaaagccacggctaactacgtgccagcagccgcggtaatacgtaggtggcaagcgttgtccggatttattgggcgtaaagcgagcgcaggcggttttttaagtctgatgtgaaagccttcggctcaaccgaagaagtgcatcggaaactgggaaacttgagtgcagaagaggacagtggaactccatgtgtagcggtgaaatgcgtagatatatggaagaacaccagtggcgaaggcggctgtctggtctgtaactgacgctgaggctcgaaagtatgggtagcaaacaggattagataccctggtagtccataccgtaaacgatgaatgctaagtgttggagggtttccgcccttcagtgctgcagctaacgcattaagcattccgcctgggagtacggccgcaaggctgaaactcaaaggaattgacgggggcccgcacaagcggtggagcatgtggtttaattcgaagctacgcgaagaaccttaccaggtcttgacatactatgcaaatctaagagattagacgttcccttcggggacatggatacaggtggtgcatggttgtcgtcagctcgtgtcgtgagatgttgggttaagtcccgcaacgagcgcaacccttattatcagttgccagcattaagttgggcactctggtgagactgccggtgacaaaccggaggaaggtgggatgacgtcaaatcatcatgccccttatgacctgggctacacacgtgctacaatggatggtacaacgagttgcgaactcgcgagagtaagctaatctcttaaagccattctcagttcggattgtaggctgcaactcgcctacatgaagtcggaatcgctagtaatcgcggatcagcatgccgcggtgaatacgttcccgggccttgtacacaccgcccgtcacaccatgagagtttgtaacacccaaagtcggtgggtaaccttttaggaaccagccgcctaaggtgggacagatgattagggtgaagtcgtaacaaggtagccgtaggagaacctgcggctggatcacct